European Patent Specification EP 3 962 909 B1, published October 4, 2023. Title: NOVEL OXALYL PIPERAZINES ACTIVE AGAINST THE HEPATITIS B VIRUS (HBV). Applicant: AiCuris GmbH & Co. KG. The sequence listing filed with the application follows.

SEQUENCE LISTING (7 sequences)

SEQ ID NO: 1 - DNA, 24 bp, Artificial Sequence
  Antisense primer HBV
tgcagaggtgaagcgaagtgcaca

SEQ ID NO: 2 - DNA, 24 bp, Artificial Sequence
  Sense primer HBV
gacgtcctttgtttacgtcccgtc

SEQ ID NO: 3 - DNA, 25 bp, Artificial Sequence
  Hybprobe FL HBV
acggggcgcacctctctttacgcgg

SEQ ID NO: 4 - DNA, 26 bp, Artificial Sequence
  Hybprobe PH HBV
ctccccgtctgtgccttctcatctgc

SEQ ID NO: 5 - DNA, 21 bp, Artificial Sequence
  HBV forward primer
ctgtaccaaaccttcggacgg

SEQ ID NO: 6 - DNA, 19 bp, Artificial Sequence
  HBV reverse primer
aggagaaacgggctgaggc

SEQ ID NO: 7 - DNA, 26 bp, Artificial Sequence
  FAM-labelled probe for HBV
ccatcatcctgggctttcggaaaatt